European Patent Specification EP 3 371 219 B1, published January 29, 2025. Title: Immunomodulatory Antibodies. Applicant: Cancer Research Technology. The sequence listing filed with the application follows.

SEQUENCE LISTING (60 sequences)

SEQ ID NO: 1 - protein, 5 aa, Artificial Sequence
  Humanised CDR
SYGVH

SEQ ID NO: 2 - protein, 8 aa, Artificial Sequence
  Humanised CDR
VIWSGGIT

SEQ ID NO: 3 - protein, 16 aa, Artificial Sequence
  Humanised CDR
NGRIGSTMTLYYAMDY

SEQ ID NO: 4 - protein, 16 aa, Artificial Sequence
  Humanised CDR
RSSKSLLHSNGITYLY

SEQ ID NO: 5 - protein, 7 aa, Artificial Sequence
  Humanised CDR
QMSNLAS

SEQ ID NO: 6 - protein, 9 aa, Artificial Sequence
  Humanised CDR
AQNLELPLT

SEQ ID NO: 7 - protein, 5 aa, Artificial Sequence
  humanised CDR
NYGVH

SEQ ID NO: 8 - protein, 8 aa, Artificial Sequence
  humanised CDR
VIWSGGST

SEQ ID NO: 9 - protein, 10 aa, Artificial Sequence
  humanised CDR
NPYYRVFMDY

SEQ ID NO: 10 - protein, 15 aa, Artificial Sequence
  humanised CDR
RASESVDSYGNSFMH

SEQ ID NO: 11 - protein, 7 aa, Artificial Sequence
  humanised CDR
RASNLES

SEQ ID NO: 12 - protein, 9 aa, Artificial Sequence
  humanised CDR
QQSNEDPFT

SEQ ID NO: 13 - protein, 5 aa, Artificial Sequence
  humanised CDR
SYGVH

SEQ ID NO: 14 - protein, 8 aa, Artificial Sequence
  humanised CDR
VIWRGGST

SEQ ID NO: 15 - protein, 11 aa, Artificial Sequence
  humanised CDR
PLGTSWDAMDY

SEQ ID NO: 16 - protein, 11 aa, Artificial Sequence
  humanised CDR
RASQDISNYLN

SEQ ID NO: 17 - protein, 7 aa, Artificial Sequence
  humanised CDR
YKSRLHS

SEQ ID NO: 18 - protein, 9 aa, Artificial Sequence
  humanised CDR
QQGNTLPYT

SEQ ID NO: 19 - protein, 10 aa, Artificial Sequence
  humanised CDR
GFSLTSYGVH

SEQ ID NO: 20 - protein, 16 aa, Artificial Sequence
  humanised CDR
VIWAGGSTNYNSALMS

SEQ ID NO: 21 - protein, 7 aa, Artificial Sequence
  humanised CDR
VREDDPY

SEQ ID NO: 22 - protein, 11 aa, Artificial Sequence
  humanised CDR
RASQDISNYLN

SEQ ID NO: 23 - protein, 7 aa, Artificial Sequence
  humanised CDR
YTSRLHS

SEQ ID NO: 24 - protein, 8 aa, Artificial Sequence
  humanised CDR
QQGNTLPF

SEQ ID NO: 25 - protein, 10 aa, Artificial Sequence
  humanised CDR
GFTFSSSYIS

SEQ ID NO: 26 - protein, 17 aa, Artificial Sequence
  humanised CDR
WIYAGTGGTSYNQKFTG

SEQ ID NO: 27 - protein, 10 aa, Artificial Sequence
  humanised CDR
ARHDYDWFAY

SEQ ID NO: 28 - protein, 12 aa, Artificial Sequence
  humanised CDR
RASSSVSSSYLH

SEQ ID NO: 29 - protein, 7 aa, Artificial Sequence
  humanised CDR
STSNLAS

SEQ ID NO: 30 - protein, 9 aa, Artificial Sequence
  humanised CDR
QQYSGYPYT

SEQ ID NO: 31 - protein, 12 aa, Artificial Sequence
  humanised CDR
GFSLSTSGKGVT

SEQ ID NO: 32 - protein, 16 aa, Artificial Sequence
  humanised CDR
TIWWDDDNRYNPSLKS

SEQ ID NO: 33 - protein, 11 aa, Artificial Sequence
  humanised CDR
VQSDWDGAMDY

SEQ ID NO: 34 - protein, 10 aa, Artificial Sequence
  humanised CDR
RASSSVSYIH

SEQ ID NO: 35 - protein, 7 aa, Artificial Sequence
  humanised CDR
ATSNLAS

SEQ ID NO: 36 - protein, 8 aa, Artificial Sequence
  humanised CDR
QQWSSHPT

SEQ ID NO: 37 - protein, 12 aa, Artificial Sequence
  humanised CDR
GFSLSTSGLGVT

SEQ ID NO: 38 - protein, 16 aa, Artificial Sequence
  humanised CDR
LIYWDDDKRYHPSLKS

SEQ ID NO: 39 - protein, 10 aa, Artificial Sequence
  humanised CDR
ARRALGTFDY

SEQ ID NO: 40 - protein, 11 aa, Artificial Sequence
  humanised CDR
RASQDISHYLN

SEQ ID NO: 41 - protein, 7 aa, Artificial Sequence
  humanised CDR
YTSRLHS

SEQ ID NO: 42 - protein, 9 aa, Artificial Sequence
  humanised CDR
QQGHTLPPT

SEQ ID NO: 43 - protein, 5 aa, Artificial Sequence
  humanised CDR
SYIMH

SEQ ID NO: 44 - protein, 17 aa, Artificial Sequence
  humanised CDR
YINPYNDNTKNNEKFKG

SEQ ID NO: 45 - protein, 11 aa, Artificial Sequence
  humanised CDR
MDYGDYPYFDY

SEQ ID NO: 46 - protein, 11 aa, Artificial Sequence
  humanised CDR
RASQDISNYLN

SEQ ID NO: 47 - protein, 7 aa, Artificial Sequence
  humanised CDR
YTSRLHS

SEQ ID NO: 48 - protein, 9 aa, Artificial Sequence
  humanised CDR
QQGNTLPFT

SEQ ID NO: 49 - protein, 5 aa, Artificial Sequence
  humanised CDR
DHYMY

SEQ ID NO: 50 - protein, 17 aa, Artificial Sequence
  humanised CDR
TISDGGRHTYYPDSVKG

SEQ ID NO: 51 - protein, 8 aa, Artificial Sequence
  humanised CDR
DLGKALDY

SEQ ID NO: 52 - protein, 11 aa, Artificial Sequence
  humanised CDR
RASENIYSNLA

SEQ ID NO: 53 - protein, 7 aa, Artificial Sequence
  humanised CDR
AATNLAD

SEQ ID NO: 54 - protein, 9 aa, Artificial Sequence
  humanised CDR
QHFWGTPWT

SEQ ID NO: 55 - protein, 5 aa, Artificial Sequence
  humanised CDR
RYIMQ

SEQ ID NO: 56 - protein, 17 aa, Artificial Sequence
  humanised CDR
YINPYNDGTRYNEKFKG

SEQ ID NO: 57 - protein, 11 aa, Artificial Sequence
  humanised CDR
FGFGDYLYFDY

SEQ ID NO: 58 - protein, 11 aa, Artificial Sequence
  humanised CDR
RASQDIRNYLN

SEQ ID NO: 59 - protein, 7 aa, Artificial Sequence
  humanised CDR
YTSRLHS

SEQ ID NO: 60 - protein, 9 aa, Artificial Sequence
  humanised CDR
QQGNTLPYT